European Patent Application EP 4 180 527 A1, published May 17, 2023. Title: SYNTHESIS METHOD OF TARGETED DRUG nCoVshRNA·2ACE2. Applicant: HANGZHOU CHICHUANG BIOTECHNOLOGY CO., LTD. The sequence listing filed with the application follows.

SEQUENCE LISTING (79 sequences)

SEQ ID NO: 1 - RNA, 30 nt, synthetic construct
  source 1..30: mol_type = other RNA
ttaatacgacctctctgttggattttgaca

SEQ ID NO: 2 - RNA, 22 nt, synthetic construct
  source 1..22: mol_type = other RNA
ggttcgcaacttcacacagagt

SEQ ID NO: 3 - RNA, 22 nt, synthetic construct
  source 1..22: mol_type = other RNA
caggcgtttgttggttgattaa

SEQ ID NO: 4 - RNA, 30 nt, synthetic construct
  source 1..30: mol_type = other RNA
gttttacgacaacgatgttggtttaggaca

SEQ ID NO: 5 - RNA, 22 nt, synthetic construct
  source 1..22: mol_type = other RNA
ggttcggttgttatatacgata

SEQ ID NO: 6 - RNA, 22 nt, synthetic construct
  source 1..22: mol_type = other RNA
ggttcagagagtctcctattta

SEQ ID NO: 7 - RNA, 21 nt, SARS-CoV-2
  source 1..21: mol_type = other RNA
gtggtattcttgctagttaca

SEQ ID NO: 8 - RNA, 21 nt, SARS-CoV-2
  source 1..21: mol_type = other RNA
ggatttgtcttctacaatttg

SEQ ID NO: 9 - RNA, 21 nt, SARS-CoV-2
  source 1..21: mol_type = other RNA
cgaacgctttcttattacaaa

SEQ ID NO: 10 - RNA, 21 nt, SARS-CoV-2
  source 1..21: mol_type = other RNA
cactgttgctacatcacgaac

SEQ ID NO: 11 - RNA, 21 nt, SARS-CoV-2
  source 1..21: mol_type = other RNA
cctagtaataggtttcctatt

SEQ ID NO: 12 - RNA, 21 nt, SARS-CoV-2
  source 1..21: mol_type = other RNA
gcgtgtagcaggtgactcagg

SEQ ID NO: 13 - RNA, 21 nt, SARS-CoV-2
  source 1..21: mol_type = other RNA
gaccgcttctagaaagtgaac

SEQ ID NO: 14 - RNA, 21 nt, SARS-CoV-2
  source 1..21: mol_type = other RNA
caaggacctgcctaaagaaat

SEQ ID NO: 15 - RNA, 21 nt, SARS-CoV-2
  source 1..21: mol_type = other RNA
atggatttgtcttctacaatt

SEQ ID NO: 16 - RNA, 21 nt, SARS-CoV-2
  source 1..21: mol_type = other RNA
cgtagtcgcaacagttcaaga

SEQ ID NO: 17 - RNA, 21 nt, SARS-CoV-2
  source 1..21: mol_type = other RNA
ggtggaccctcagattcaact

SEQ ID NO: 18 - RNA, 21 nt, SARS-CoV-2
  source 1..21: mol_type = other RNA
ggttcaccgctctcactcaac

SEQ ID NO: 19 - RNA, 21 nt, SARS-CoV-2
  source 1..21: mol_type = other RNA
cgggaacgtggttgacctaca

SEQ ID NO: 20 - RNA, 21 nt, SARS-CoV-2
  source 1..21: mol_type = other RNA
gcttatgtgtcaacctatact

SEQ ID NO: 21 - RNA, 21 nt, SARS-CoV-2
  source 1..21: mol_type = other RNA
ggttgaagcagttaattaaag

SEQ ID NO: 22 - RNA, 21 nt, SARS-CoV-2
  source 1..21: mol_type = other RNA
cgatattacgcacaactaatg

SEQ ID NO: 23 - RNA, 21 nt, SARS-CoV-2
  source 1..21: mol_type = other RNA
agaccatgttgacatactagg

SEQ ID NO: 24 - RNA, 21 nt, SARS-CoV-2
  source 1..21: mol_type = other RNA
ggttctttaatctactcaacc

SEQ ID NO: 25 - RNA, 21 nt, SARS-CoV-2
  source 1..21: mol_type = other RNA
ggtggtgttgttcagttgact

SEQ ID NO: 26 - RNA, 21 nt, SARS-CoV-2
  source 1..21: mol_type = other RNA
gctcgtgttgtacgatcaatt

SEQ ID NO: 27 - RNA, 21 nt, SARS-CoV-2
  source 1..21: mol_type = other RNA
agtgtataatgctagtttatt

SEQ ID NO: 28 - RNA, 21 nt, SARS-CoV-2
  source 1..21: mol_type = other RNA
ggtacatgtcagcattaaatc

SEQ ID NO: 29 - RNA, 21 nt, SARS-CoV-2
  source 1..21: mol_type = other RNA
gttagatgatgatagtcaaca

SEQ ID NO: 30 - RNA, 21 nt, SARS-CoV-2
  source 1..21: mol_type = other RNA
gattgtttaggaagtctaatc

SEQ ID NO: 31 - RNA, 21 nt, SARS-CoV-2
  source 1..21: mol_type = other RNA
gtctctagtcagtgtgttaat

SEQ ID NO: 32 - RNA, 21 nt, SARS-CoV-2
  source 1..21: mol_type = other RNA
ctactaatgttgttattaaag

SEQ ID NO: 33 - RNA, 21 nt, SARS-CoV-2
  source 1..21: mol_type = other RNA
ggtgttcttactgagtctaac

SEQ ID NO: 34 - RNA, 21 nt, SARS-CoV-2
  source 1..21: mol_type = other RNA
gaaacaaagtgtacgttgaaa

SEQ ID NO: 35 - RNA, 21 nt, SARS-CoV-2
  source 1..21: mol_type = other RNA
gttagatttcctaatattaca

SEQ ID NO: 36 - RNA, 21 nt, SARS-CoV-2
  source 1..21: mol_type = other RNA
ctgtgatgttgtaataggaat

SEQ ID NO: 37 - RNA, 21 nt, SARS-CoV-2
  source 1..21: mol_type = other RNA
ggagtcaaattacattacaca

SEQ ID NO: 38 - RNA, 21 nt, SARS-CoV-2
  source 1..21: mol_type = other RNA
gcttactctaataactctatt

SEQ ID NO: 39 - RNA, 21 nt, SARS-CoV-2
  source 1..21: mol_type = other RNA
ggtaactgtgatgttgtaata

SEQ ID NO: 40 - RNA, 21 nt, SARS-CoV-2
  source 1..21: mol_type = other RNA
tggtaactgtgatgttgtaat

SEQ ID NO: 41 - RNA, 21 nt, SARS-CoV-2
  source 1..21: mol_type = other RNA
ggtacgttaatagttaatagc

SEQ ID NO: 42 - RNA, 21 nt, SARS-CoV-2
  source 1..21: mol_type = other RNA
gtggtattcttgctagttaca

SEQ ID NO: 43 - RNA, 21 nt, SARS-CoV-2
  source 1..21: mol_type = other RNA
gttaatagttaatagcgtact

SEQ ID NO: 44 - RNA, 21 nt, SARS-CoV-2
  source 1..21: mol_type = other RNA
ggtggaattgctatcgcaatg

SEQ ID NO: 45 - RNA, 21 nt, SARS-CoV-2
  source 1..21: mol_type = other RNA
ggatttgtcttctacaatttg

SEQ ID NO: 46 - RNA, 21 nt, SARS-CoV-2
  source 1..21: mol_type = other RNA
cgaacgctttcttattacaaa

SEQ ID NO: 47 - RNA, 21 nt, SARS-CoV-2
  source 1..21: mol_type = other RNA
cactgttgctacatcacgaac

SEQ ID NO: 48 - RNA, 21 nt, SARS-CoV-2
  source 1..21: mol_type = other RNA
cctagtaataggtttcctatt

SEQ ID NO: 49 - RNA, 21 nt, SARS-CoV-2
  source 1..21: mol_type = other RNA
cgtagtcgcaacagttcaaga

SEQ ID NO: 50 - RNA, 21 nt, SARS-CoV-2
  source 1..21: mol_type = other RNA
ggctactaccgaagagctacc

SEQ ID NO: 51 - RNA, 21 nt, SARS-CoV-2
  source 1..21: mol_type = other RNA
caagatggtatttctactacc

SEQ ID NO: 52 - RNA, 21 nt, SARS-CoV-2
  source 1..21: mol_type = other RNA
gcttatgtgtcaacctatact

SEQ ID NO: 53 - RNA, 21 nt, SARS-CoV-2
  source 1..21: mol_type = other RNA
ggttgaagcagttaattaaag

SEQ ID NO: 54 - RNA, 21 nt, SARS-CoV-2
  source 1..21: mol_type = other RNA
cgatattacgcacaactaatg

SEQ ID NO: 55 - RNA, 21 nt, SARS-CoV-2
  source 1..21: mol_type = other RNA
gattgtttaggaagtctaatc

SEQ ID NO: 56 - RNA, 21 nt, SARS-CoV-2
  source 1..21: mol_type = other RNA
gtctctagtcagtgtgttaat

SEQ ID NO: 57 - RNA, 21 nt, SARS-CoV-2
  source 1..21: mol_type = other RNA
ctactaatgttgttattaaag

SEQ ID NO: 58 - RNA, 21 nt, SARS-CoV-2
  source 1..21: mol_type = other RNA
ggtgttcttactgagtctaac

SEQ ID NO: 59 - protein, 740 aa, human
MSSSSWLLLSLVAVTAAQSTIEEQAKTFLDKFNHEAEDLFYQSSLASWNYNTNITEENVQNMNNAGDKWSAFLKEQSTLAQMYPLQEIQNLTVKLQLQALQQNGSSVLSEDKSKRLNTILNTMSTIYSTGKVCNPDNPQECLLLEPGLNEIMANSLDYNERLWAWESWRSEVGKQLRPLYEEYVVLKNEMARANHYEDYGDYWRGDYEVNGVDGYDYSRGQLIEDVEHTFEEIKPLYEHLHAYVRAKLMNAYPSYISPIGCLPAHLLGDMWGRFWTNLYSLTVPFGQKPNIDVTDAMVDQAWDAQRIFKEAEKFFVSVGLPNMTQGFWENSMLTDPGNVQKAVCHPTAWDLGKGDFRILMCTKVTMDDFLTAHHEMGHIQYDMAYAAQPFLLRNGANEGFHEAVGEIMSLSAATPKHLKSIGLLSPDFQEDNETEINFLLKQALTIVGTLPFTYMLEKWRWMVFKGEIPKDQWMKKWWEMKREIVGVVEPVPHDETYCDPASLFHVSNDYSFIRYYTRTLYQFQFQEALCQAAKHEGPLHKCDISNSTEAGQKLFNMLRLGKSEPWTLALENVVGAKNMNVRPLLNYFEPLFTWLKDQNKNSFVGWSTDWSPYADQSIKVRISLKSALGDKAYEWNDNEMYLFRSSVAYAMRQYFLKVKNQMILFGEEDVRVANLKPRISFNFFVTAPKNVSDIIPRTEVEKAIRMSRSRINDAFRLNDNSLEFLGIQPTLGPPNQPPVS

SEQ ID NO: 60 - protein, 23 aa, human
IWLIVFGVVMGVIVVGIVILIFT

SEQ ID NO: 61 - protein, 42 aa, human
GIRDRKKKNKARSGENPYASIDISKGENNPGFQNTDDVQTSF

SEQ ID NO: 62 - RNA, 21 nt, SARS-CoV-2
  source 1..21: mol_type = other RNA
ggaagagacaggtacgttaat

SEQ ID NO: 63 - RNA, 21 nt, SARS-CoV-2
  source 1..21: mol_type = other RNA
gaagagacaggtacgttaata

SEQ ID NO: 64 - RNA, 21 nt, SARS-CoV-2
  source 1..21: mol_type = other RNA
gctgctgtttacagaataaat

SEQ ID NO: 65 - RNA, 21 nt, SARS-CoV-2
  source 1..21: mol_type = other RNA
cggtactattaccgttgaaga

SEQ ID NO: 66 - RNA, 21 nt, SARS-CoV-2
  source 1..21: mol_type = other RNA
ggttccaacggtactattacc

SEQ ID NO: 67 - RNA, 21 nt, SARS-CoV-2
  source 1..21: mol_type = other RNA
cgaagagctaccagacgaatt

SEQ ID NO: 68 - RNA, 21 nt, SARS-CoV-2
  source 1..21: mol_type = other RNA
gagacagaagaaacagcaaac

SEQ ID NO: 69 - RNA, 21 nt, SARS-CoV-2
  source 1..21: mol_type = other RNA
ggatgatttctccaaacaatt

SEQ ID NO: 70 - RNA, 21 nt, SARS-CoV-2
  source 1..21: mol_type = other RNA
ggacgaagatgacaatttaat

SEQ ID NO: 71 - RNA, 21 nt, SARS-CoV-2
  source 1..21: mol_type = other RNA
ggtgttgtttgtacagaaatt

SEQ ID NO: 72 - RNA, 21 nt, SARS-CoV-2
  source 1..21: mol_type = other RNA
cctcagtgttgacactaaatt

SEQ ID NO: 73 - RNA, 21 nt, SARS-CoV-2
  source 1..21: mol_type = other RNA
ggatgttaactgcacagaagt

SEQ ID NO: 74 - RNA, 21 nt, SARS-CoV-2
  source 1..21: mol_type = other RNA
gcaactgtgttgctgattatt

SEQ ID NO: 75 - RNA, 21 nt, SARS-CoV-2
  source 1..21: mol_type = other RNA
gggtgttaactgcacagaagt

SEQ ID NO: 76 - RNA, 21 nt, SARS-CoV-2
  source 1..21: mol_type = other RNA
ggtatagattgtttaggaagt

SEQ ID NO: 77 - RNA, 68 nt, synthetic construct
  source 1..68: mol_type = other RNA
ttaatacgacctctctgttggattttgacattcaagagatgtcaaatccaacagagaggtcgtattaa

SEQ ID NO: 78 - RNA, 53 nt, synthetic construct
  source 1..53: mol_type = other RNA
ggttcgcaacttcacacagagtttcaagagaactctgtgtgaagttgcgaacc

SEQ ID NO: 79 - RNA, 53 nt, synthetic construct
  source 1..53: mol_type = other RNA
ggttcggttgttatatacgatattcaagagatatcgtatataacaaccgaacc